European Patent Application EP 4 190 807 A1, published June 7, 2023. Title: TRUNCATED BODY OF IL7Rα AND USE THEREOF IN PREPARATION OF MEDICATION FOR TREATING TUMOR. Applicant: Beijing Neurosurgical Institute. The sequence listing filed with the application follows.

SEQUENCE LISTING (8 sequences)

SEQ ID NO: 1 - protein, 95 aa, Artificial Sequence
  This sequence is synthesized in lab.
KKRIKPIVWPSLPDHKKTLEHLCKKPRKNLNVSFNPESFLDCQIHRVDDIQARDEVEGFLQDTFPQQLEESEKQRLLGSNQEEAYVTMSSFYQNQ

SEQ ID NO: 2 - DNA, 285 bp, Artificial Sequence
  This sequence is synthesized in lab.
aaaaaaaggattaagcctatcgtatggcccagtctccccgatcacaagaagactctggaacacctttgtaagaaaccaagaaaaaatttaaatgtgagtttcaatcctgaaagtttcctggactgccagattcatagggtggatgacattcaagctagagatgaagtggaaggttttctgcaagatacgtttcctcagcaactagaagaatctgagaagcagaggcttctgggatcaaatcaagaagaagcatatgtcaccatgtccagcttctaccaaaaccag

SEQ ID NO: 3 - protein, 822 aa, Artificial Sequence
  This sequence is synthesized in lab.
QVQLVESGGGVVQPGRSLRLSCAASGFTFSSYGMHWVRQAPGKGLEWVAVIWYDGSNKFYADSVKGRFTISRDNSKNTLYLQMNSLRAEDTAVYYCARRSDYRGYYGMDVWGQGTTVTVSSGSTSGGGSGGGSGGGGSSEIVLTQSPATLSLSPGERATLSCRASQSVINYLAWYQQKPGQAPRLLIYDASNRASGIPARFSGSGSGTDFTLTISSLEPEDFAVYYCQQRRNWPLTFGGGTKVEIKGGGGSGGGGSGGGGSQVQLVQSGAEVKKPGASVKVSCKASGYTFTDFEMHWVRQAPGQGLEWMGDIDPGTGDTAYNLKFKGRVTMTTDTSTSTAYMELRSLRSDDTAVYYCALGAFVYWGQGTLVTVSSGSTSGGGSGGGSGGGGSSDVVMTQSPLSLPVTPGEPASISCRSSQSLANSYGNTYLSWYLQKPGQSPQLLIYGISNRFSGVPDRFSGSGSGTDFTLKISRVEAEDVGVYYCLQGTHQPYTFGQGTKLEIKTTTPAPRPPTPAPTIASQPLSLRPEACRPAAGGAVHTRGLDFACDIYIWAPLAGTCGVLLLSLVITLYCRSKRSRLLHSDYMNMTPRRPGPTRKHYQPYAPPRDFAAYRSKKRIKPIVWPSLPDHKKTLEHLCKKPRKNLNVSFNPESFLDCQIHRVDDIQARDEVEGFLQDTFPQQLEESEKQRLLGSNQEEAYVTMSSFYQNQRVKFSRSADAPAYKQGQNQLYNELNLGRREEYDVLDKRRGRDPEMGGKPRRKNPQEGLYNELQKDKMAEAYSEIGMKGERRRGKGHDGLYQGLSTATKDTYDALHMQALPPR

SEQ ID NO: 4 - DNA, 2466 bp, Artificial Sequence
  This sequence is synthesized in lab.
caggtgcagctggtggagtctgggggaggcgtggtccagcctgggaggtccctgagactctcctgtgcagcgtctggattcaccttcagtagctatggcatgcactgggtccgccaggctccaggcaaggggctggagtgggtggcagttatatggtatgatggaagtaataaattctatgcagactccgtgaagggccgattcaccatctccagagacaattccaagaacacgctgtatctgcaaatgaacagcctgagagccgaggacacggctgtgtattactgtgcgaggagaagtgactacaggggctactacggtatggacgtctggggccaagggaccacggtcaccgtctcctcaggcagtactagcggtggtggctccgggggcggttccggtgggggcggcagcagcgaaattgtgttgacacagtctccagccaccctgtctttgtctccaggggaaagagccaccctctcctgcagggccagtcagagtgttatcaactacttagcctggtaccaacagaaacctggccaggctcccaggctcctcatctatgatgcatccaacagggcctctggcatcccagccaggttcagtggcagtgggtctgggacagacttcactctcaccatcagcagcctagagcctgaagattttgcagtttattactgtcagcagcgtcgcaactggccgctcactttcggcggagggaccaaggtggagatcaaaggaggtggtggatccggaggtggtggctccggaggtggtggatcccaggttcagctggtgcagtctggagctgaggtgaagaagcctggggcctcagtgaaggtctcctgcaaggcttctggttacacctttaccgactttgaaatgcactgggtgcgacaggcccctggacaagggcttgagtggatgggagatattgatcctggaactggtgatactgcctacaatctgaagttcaagggcagagtcaccatgaccacagacacatccacgagcacagcctacatggagctgaggagcctgaggtctgacgacacggccgtgtattactgtgcgttgggggcctttgtttactggggccagggaaccctggtcaccgtctcctcaggcagtactagcggtggtggctccgggggcggttccggtgggggcggcagcagcgatgttgtgatgactcagtctccactctccctgcccgtcacccctggagagccggcctccatctcctgcaggtctagtcagagtcttgcaaacagttatgggaacacctatttgtcttggtacctgcagaagccagggcagtctccacagctcctgatctatgggatttccaacagattttctggggtccctgacaggttcagtggcagtggatcaggcacagattttacactgaaaatcagcagagtggaggctgaggacgttggggtttattactgcttacaaggtacacatcagccgtacacgtttggccaggggaccaagctggagatcaaaaccactaccccagcaccgaggccacccaccccggctcctaccatcgcctcccagcctctgtccctgcgtccggaggcatgtagacccgcagctggtggggccgtgcatacccggggtcttgacttcgcctgcgatatctacatttgggcccctctggctggtacttgcggggtcctgctgctttcactcgtgatcactctttactgtaggagtaagaggagcaggctcctgcacagtgactacatgaacatgactccccgccgccccgggcccacccgcaagcattaccagccctatgccccaccacgcgacttcgcagcctatcgctccaaaaaaaggattaagcctatcgtatggcccagtctccccgatcacaagaagactctggaacacctttgtaagaaaccaagaaaaaatttaaatgtgagtttcaatcctgaaagtttcctggactgccagattcatagggtggatgacattcaagctagagatgaagtggaaggttttctgcaagatacgtttcctcagcaactagaagaatctgagaagcagaggcttctgggatcaaatcaagaagaagcatatgtcaccatgtccagcttctaccaaaaccagcgcgtgaaattcagccgcagcgcagatgctccagcctacaagcaggggcagaaccagctctacaacgaactcaatcttggtcggagagaggagtacgacgtgctggacaagcggagaggacgggacccagaaatgggcgggaagccgcgcagaaagaatccccaagagggcctgtacaacgagctccaaaaggataagatggcagaagcctatagcgagattggtatgaaaggggaacgcagaagaggcaaaggccacgacggactgtaccagggactcagcaccgccaccaaggacacctatgacgctcttcacatgcaggccctgccgcctcgg

SEQ ID NO: 5 - DNA, 2181 bp, Artificial Sequence
  This sequence is synthesized in lab.
caggtgcagctggtggagtctgggggaggcgtggtccagcctgggaggtccctgagactctcctgtgcagcgtctggattcaccttcagtagctatggcatgcactgggtccgccaggctccaggcaaggggctggagtgggtggcagttatatggtatgatggaagtaataaattctatgcagactccgtgaagggccgattcaccatctccagagacaattccaagaacacgctgtatctgcaaatgaacagcctgagagccgaggacacggctgtgtattactgtgcgaggagaagtgactacaggggctactacggtatggacgtctggggccaagggaccacggtcaccgtctcctcaggcagtactagcggtggtggctccgggggcggttccggtgggggcggcagcagcgaaattgtgttgacacagtctccagccaccctgtctttgtctccaggggaaagagccaccctctcctgcagggccagtcagagtgttatcaactacttagcctggtaccaacagaaacctggccaggctcccaggctcctcatctatgatgcatccaacagggcctctggcatcccagccaggttcagtggcagtgggtctgggacagacttcactctcaccatcagcagcctagagcctgaagattttgcagtttattactgtcagcagcgtcgcaactggccgctcactttcggcggagggaccaaggtggagatcaaaggaggtggtggatccggaggtggtggctccggaggtggtggatcccaggttcagctggtgcagtctggagctgaggtgaagaagcctggggcctcagtgaaggtctcctgcaaggcttctggttacacctttaccgactttgaaatgcactgggtgcgacaggcccctggacaagggcttgagtggatgggagatattgatcctggaactggtgatactgcctacaatctgaagttcaagggcagagtcaccatgaccacagacacatccacgagcacagcctacatggagctgaggagcctgaggtctgacgacacggccgtgtattactgtgcgttgggggcctttgtttactggggccagggaaccctggtcaccgtctcctcaggcagtactagcggtggtggctccgggggcggttccggtgggggcggcagcagcgatgttgtgatgactcagtctccactctccctgcccgtcacccctggagagccggcctccatctcctgcaggtctagtcagagtcttgcaaacagttatgggaacacctatttgtcttggtacctgcagaagccagggcagtctccacagctcctgatctatgggatttccaacagattttctggggtccctgacaggttcagtggcagtggatcaggcacagattttacactgaaaatcagcagagtggaggctgaggacgttggggtttattactgcttacaaggtacacatcagccgtacacgtttggccaggggaccaagctggagatcaaaaccactaccccagcaccgaggccacccaccccggctcctaccatcgcctcccagcctctgtccctgcgtccggaggcatgtagacccgcagctggtggggccgtgcatacccggggtcttgacttcgcctgcgatatctacatttgggcccctctggctggtacttgcggggtcctgctgctttcactcgtgatcactctttactgtaggagtaagaggagcaggctcctgcacagtgactacatgaacatgactccccgccgccccgggcccacccgcaagcattaccagccctatgccccaccacgcgacttcgcagcctatcgctcccgcgtgaaattcagccgcagcgcagatgctccagcctacaagcaggggcagaaccagctctacaacgaactcaatcttggtcggagagaggagtacgacgtgctggacaagcggagaggacgggacccagaaatgggcgggaagccgcgcagaaagaatccccaagagggcctgtacaacgagctccaaaaggataagatggcagaagcctatagcgagattggtatgaaaggggaacgcagaagaggcaaaggccacgacggactgtaccagggactcagcaccgccaccaaggacacctatgacgctcttcacatgcaggccctgccgcctcgg

SEQ ID NO: 6 - DNA, 2766 bp, Artificial Sequence
  This sequence is synthesized in lab.
caggtgcagctggtggagtctgggggaggcgtggtccagcctgggaggtccctgagactctcctgtgcagcgtctggattcaccttcagtagctatggcatgcactgggtccgccaggctccaggcaaggggctggagtgggtggcagttatatggtatgatggaagtaataaattctatgcagactccgtgaagggccgattcaccatctccagagacaattccaagaacacgctgtatctgcaaatgaacagcctgagagccgaggacacggctgtgtattactgtgcgaggagaagtgactacaggggctactacggtatggacgtctggggccaagggaccacggtcaccgtctcctcaggcagtactagcggtggtggctccgggggcggttccggtgggggcggcagcagcgaaattgtgttgacacagtctccagccaccctgtctttgtctccaggggaaagagccaccctctcctgcagggccagtcagagtgttatcaactacttagcctggtaccaacagaaacctggccaggctcccaggctcctcatctatgatgcatccaacagggcctctggcatcccagccaggttcagtggcagtgggtctgggacagacttcactctcaccatcagcagcctagagcctgaagattttgcagtttattactgtcagcagcgtcgcaactggccgctcactttcggcggagggaccaaggtggagatcaaaggaggtggtggatccggaggtggtggctccggaggtggtggatcccaggttcagctggtgcagtctggagctgaggtgaagaagcctggggcctcagtgaaggtctcctgcaaggcttctggttacacctttaccgactttgaaatgcactgggtgcgacaggcccctggacaagggcttgagtggatgggagatattgatcctggaactggtgatactgcctacaatctgaagttcaagggcagagtcaccatgaccacagacacatccacgagcacagcctacatggagctgaggagcctgaggtctgacgacacggccgtgtattactgtgcgttgggggcctttgtttactggggccagggaaccctggtcaccgtctcctcaggcagtactagcggtggtggctccgggggcggttccggtgggggcggcagcagcgatgttgtgatgactcagtctccactctccctgcccgtcacccctggagagccggcctccatctcctgcaggtctagtcagagtcttgcaaacagttatgggaacacctatttgtcttggtacctgcagaagccagggcagtctccacagctcctgatctatgggatttccaacagattttctggggtccctgacaggttcagtggcagtggatcaggcacagattttacactgaaaatcagcagagtggaggctgaggacgttggggtttattactgcttacaaggtacacatcagccgtacacgtttggccaggggaccaagctggagatcaaaaccactaccccagcaccgaggccacccaccccggctcctaccatcgcctcccagcctctgtccctgcgtccggaggcatgtagacccgcagctggtggggccgtgcatacccggggtcttgacttcgcctgcgatatctacatttgggcccctctggctggtacttgcggggtcctgctgctttcactcgtgatcactctttactgtaggagtaagaggagcaggctcctgcacagtgactacatgaacatgactccccgccgccccgggcccacccgcaagcattaccagccctatgccccaccacgcgacttcgcagcctatcgctccaaaaaaaggattaagcctatcgtatggcccagtctccccgatcataagaagactctggaacatctttgtaagaaaccaagaaaaaatttaaatgtgagtttcaatcctgaaagtttcctggactgccagattcatagggtggatgacattcaagctagagatgaagtggaaggttttctgcaagatacgtttcctcagcaactagaagaatctgagaagcagaggcttggaggggatgtgcagagccccaactgcccatctgaggatgtagtcatcactccagaaagctttggaagagattcatccctcacatgcctggctgggaatgtcagtgcatgtgacgcccctattctctccccttccaggtccctagactgcagggagagtggcaagaatgggcctcatgtgtaccaggacctcctgcttagccttgggactacaaacagcacgctgccccctccattttctctccaatctggaatcctgacattgaacccagttgctcagggtcagcccattcttacttccctgggatcaaatcaagaagaagcatatgtcaccatgtccagcttctaccaaaaccagcgcgtgaaattcagccgcagcgcagatgctccagcctacaagcaggggcagaaccagctctacaacgaactcaatcttggtcggagagaggagtacgacgtgctggacaagcggagaggacgggacccagaaatgggcgggaagccgcgcagaaagaatccccaagagggcctgtacaacgagctccaaaaggataagatggcagaagcctatagcgagattggtatgaaaggggaacgcagaagaggcaaaggccacgacggactgtaccagggactcagcaccgccaccaaggacacctatgacgctcttcacatgcaggccctgccgcctcgg

SEQ ID NO: 7 - protein, 727 aa, Artificial Sequence
  This sequence is synthesized in lab.
QVQLVESGGGVVQPGRSLRLSCAASGFTFSSYGMHWVRQAPGKGLEWVAVIWYDGSNKFYADSVKGRFTISRDNSKNTLYLQMNSLRAEDTAVYYCARRSDYRGYYGMDVWGQGTTVTVSSGSTSGGGSGGGSGGGGSSEIVLTQSPATLSLSPGERATLSCRASQSVINYLAWYQQKPGQAPRLLIYDASNRASGIPARFSGSGSGTDFTLTISSLEPEDFAVYYCQQRRNWPLTFGGGTKVEIKGGGGSGGGGSGGGGSQVQLVQSGAEVKKPGASVKVSCKASGYTFTDFEMHWVRQAPGQGLEWMGDIDPGTGDTAYNLKFKGRVTMTTDTSTSTAYMELRSLRSDDTAVYYCALGAFVYWGQGTLVTVSSGSTSGGGSGGGSGGGGSSDVVMTQSPLSLPVTPGEPASISCRSSQSLANSYGNTYLSWYLQKPGQSPQLLIYGISNRFSGVPDRFSGSGSGTDFTLKISRVEAEDVGVYYCLQGTHQPYTFGQGTKLEIKTTTPAPRPPTPAPTIASQPLSLRPEACRPAAGGAVHTRGLDFACDIYIWAPLAGTCGVLLLSLVITLYCRSKRSRLLHSDYMNMTPRRPGPTRKHYQPYAPPRDFAAYRSRVKFSRSADAPAYKQGQNQLYNELNLGRREEYDVLDKRRGRDPEMGGKPRRKNPQEGLYNELQKDKMAEAYSEIGMKGERRRGKGHDGLYQGLSTATKDTYDALHMQALPPR

SEQ ID NO: 8 - protein, 921 aa, Artificial Sequence
  This sequence is synthesized in lab.
QVQLVESGGGVVQPGRSLRLSCAASGFTFSSYGMHWVRQAPGKGLEWVAVIWYDGSNKFYADSVKGRFTISRDNSKNTLYLQMNSLRAEDTAVYYCARRSDYRGYYGMDVWGQGTTVTVSSGSTSGGGSGGGSGGGGSSEIVLTQSPATLSLSPGERATLSCRASQSVINYLAWYQQKPGQAPRLLIYDASNRASGIPARFSGSGSGTDFTLTISSLEPEDFAVYYCQQRRNWPLTFGGGTKVEIKGGGGSGGGGSGGGGSQVQLVQSGAEVKKPGASVKVSCKASGYTFTDFEMHWVRQAPGQGLEWMGDIDPGTGDTAYNLKFKGRVTMTTDTSTSTAYMELRSLRSDDTAVYYCALGAFVYWGQGTLVTVSSGSTSGGGSGGGSGGGGSSDVVMTQSPLSLPVTPGEPASISCRSSQSLANSYGNTYLSWYLQKPGQSPQLLIYGISNRFSGVPDRFSGSGSGTDFTLKISRVEAEDVGVYYCLQGTHQPYTFGQGTKLEIKTTTPAPRPPTPAPTIASQPLSLRPEACRPAAGGAVHTRGLDFACDIYIWAPLAGTCGVLLLSLVITLYCRSKRSRLLHSDYMNMTPRRPGPTRKHYQPYAPPRDFAAYRSKKRIKPIVWPSLPDHKKTLEHLCKKPRKNLNVSFNPESFLDCQIHRVDDIQARDEVEGFLQDTFPQQLEESEKQRLGGDVQSPNCPSEDVVITPESFGRDSSLTCLAGNVSACDAPILSPSRSLDCRESGKNGPHVYQDLLLSLGTTNSTLPPPFSLQSGILTLNPVAQGQPILTSLGSNQEEAYVTMSSFYQNQRVKFSRSADAPAYKQGQNQLYNELNLGRREEYDVLDKRRGRDPEMGGKPRKNPQEGLYNELQKDKMAEAYSEIGMKGERRRGKGHDGLYQGLSTATKDTYDALHMQALPPR